European Patent Application EP 4 602 916 A1, published August 20, 2025. Title: A composition for increasing stres resistance in plants. Applicant: KIRIN HOLDINGS KABUSHIKI KAISHA. The sequence listing filed with the application follows.

SEQUENCE LISTING (46 sequences)

SEQ ID NO: 1 - DNA, 20 bp, synthetic construct
  misc_feature 1..20: note = Primer
  source 1..20: mol_type = other DNA
atcagcaaggatctgggatg

SEQ ID NO: 2 - DNA, 20 bp, synthetic construct
  misc_feature 1..20: note = Primer
  source 1..20: mol_type = other DNA
cctcagctacaagcacacca

SEQ ID NO: 3 - DNA, 20 bp, synthetic construct
  misc_feature 1..20: note = Primer
  source 1..20: mol_type = other DNA
caaaacagagcaaacgcaaa

SEQ ID NO: 4 - DNA, 20 bp, synthetic construct
  misc_feature 1..20: note = Primer
  source 1..20: mol_type = other DNA
aacgcatcgaaaacatccag

SEQ ID NO: 5 - DNA, 22 bp, synthetic construct
  misc_feature 1..22: note = Primer
  source 1..22: mol_type = other DNA
gatctccaaggccgagtatgat

SEQ ID NO: 6 - DNA, 20 bp, synthetic construct
  misc_feature 1..20: note = Primer
  source 1..20: mol_type = other DNA
cccattcataaaaccccagc

SEQ ID NO: 7 - DNA, 21 bp, synthetic construct
  misc_feature 1..21: note = Primer
  source 1..21: mol_type = other DNA
cacaaagtcagacctgcaagc

SEQ ID NO: 8 - DNA, 20 bp, synthetic construct
  misc_feature 1..20: note = Primer
  source 1..20: mol_type = other DNA
atgccatcatgtgctgttgc

SEQ ID NO: 9 - DNA, 20 bp, synthetic construct
  misc_feature 1..20: note = Primer
  source 1..20: mol_type = other DNA
agcacattccagcagatgtg

SEQ ID NO: 10 - DNA, 20 bp, synthetic construct
  misc_feature 1..20: note = Primer
  source 1..20: mol_type = other DNA
ttcctgtgcacaatggatgg

SEQ ID NO: 11 - DNA, 20 bp, synthetic construct
  misc_feature 1..20: note = Primer
  source 1..20: mol_type = other DNA
tcgcgaacaaagggtttcag

SEQ ID NO: 12 - DNA, 20 bp, synthetic construct
  misc_feature 1..20: note = Primer
  source 1..20: mol_type = other DNA
accggattttgcagaatcgg

SEQ ID NO: 13 - DNA, 20 bp, synthetic construct
  misc_feature 1..20: note = Primer
  source 1..20: mol_type = other DNA
tgctcgcattgactggaaag

SEQ ID NO: 14 - DNA, 22 bp, synthetic construct
  misc_feature 1..22: note = Primer
  source 1..22: mol_type = other DNA
ttgtcctccttctccacattcc

SEQ ID NO: 15 - DNA, 20 bp, synthetic construct
  misc_feature 1..20: note = Primer
  source 1..20: mol_type = other DNA
ttttgctgtcagggacatgc

SEQ ID NO: 16 - DNA, 20 bp, synthetic construct
  misc_feature 1..20: note = Primer
  source 1..20: mol_type = other DNA
ttggcagcggatttggtaac

SEQ ID NO: 17 - DNA, 20 bp, synthetic construct
  misc_feature 1..20: note = Primer
  source 1..20: mol_type = other DNA
gcttctccgattcctccttt

SEQ ID NO: 18 - DNA, 20 bp, synthetic construct
  misc_feature 1..20: note = Primer
  source 1..20: mol_type = other DNA
gaccaccgagagcttggtaa

SEQ ID NO: 19 - DNA, 20 bp, synthetic construct
  misc_feature 1..20: note = Primer
  source 1..20: mol_type = other DNA
ggcgaattgtttgatgcttt

SEQ ID NO: 20 - DNA, 20 bp, synthetic construct
  misc_feature 1..20: note = Primer
  source 1..20: mol_type = other DNA
caagccactctcttcccact

SEQ ID NO: 21 - DNA, 23 bp, synthetic construct
  misc_feature 1..23: note = Primer
  source 1..23: mol_type = other DNA
gaccaagtgaaccaggttattgg

SEQ ID NO: 22 - DNA, 22 bp, synthetic construct
  misc_feature 1..22: note = Primer
  source 1..22: mol_type = other DNA
tactctccagtgcctgtcttca

SEQ ID NO: 23 - DNA, 19 bp, synthetic construct
  misc_feature 1..19: note = Primer
  source 1..19: mol_type = other DNA
acgacgacgacgaagaacg

SEQ ID NO: 24 - DNA, 20 bp, synthetic construct
  misc_feature 1..20: note = Primer
  source 1..20: mol_type = other DNA
ttcaagtccaggcagacacc

SEQ ID NO: 25 - DNA, 20 bp, synthetic construct
  misc_feature 1..20: note = Primer
  source 1..20: mol_type = other DNA
agcacattccagcagatgtg

SEQ ID NO: 26 - DNA, 20 bp, synthetic construct
  misc_feature 1..20: note = Primer
  source 1..20: mol_type = other DNA
ttcctgtgcacaatggatgg

SEQ ID NO: 27 - DNA, 22 bp, synthetic construct
  misc_feature 1..22: note = Primer
  source 1..22: mol_type = other DNA
caattctccaaccacggctaac

SEQ ID NO: 28 - DNA, 21 bp, synthetic construct
  misc_feature 1..21: note = Primer
  source 1..21: mol_type = other DNA
atggctcgtggaattggagag

SEQ ID NO: 29 - DNA, 22 bp, synthetic construct
  misc_feature 1..22: note = Primer
  source 1..22: mol_type = other DNA
cctggacatggctaattgcttg

SEQ ID NO: 30 - DNA, 20 bp, synthetic construct
  misc_feature 1..20: note = Primer
  source 1..20: mol_type = other DNA
aagtcttgcaagcgaacacg

SEQ ID NO: 31 - DNA, 20 bp, synthetic construct
  misc_feature 1..20: note = Primer
  source 1..20: mol_type = other DNA
ttttgctgtcagggacatgc

SEQ ID NO: 32 - DNA, 20 bp, synthetic construct
  misc_feature 1..20: note = Primer
  source 1..20: mol_type = other DNA
ttggcagcggatttggtaac

SEQ ID NO: 33 - DNA, 22 bp, synthetic construct
  misc_feature 1..22: note = Primer
  source 1..22: mol_type = other DNA
ttcagtcttccatggagtcgag

SEQ ID NO: 34 - DNA, 22 bp, synthetic construct
  misc_feature 1..22: note = Primer
  source 1..22: mol_type = other DNA
gaggttttggtggtggaaatcg

SEQ ID NO: 35 - DNA, 22 bp, synthetic construct
  misc_feature 1..22: note = Primer
  source 1..22: mol_type = other DNA
tgcgatatcggagatcaagtcg

SEQ ID NO: 36 - DNA, 20 bp, synthetic construct
  misc_feature 1..20: note = Primer
  source 1..20: mol_type = other DNA
ttttgatcgccaccgtcaac

SEQ ID NO: 37 - DNA, 21 bp, synthetic construct
  misc_feature 1..21: note = Primer
  source 1..21: mol_type = other DNA
tccacgcctcaatctctcaac

SEQ ID NO: 38 - DNA, 22 bp, synthetic construct
  misc_feature 1..22: note = Primer
  source 1..22: mol_type = other DNA
tgggttttgggtaaagtttgcg

SEQ ID NO: 39 - DNA, 20 bp, synthetic construct
  misc_feature 1..20: note = Primer
  source 1..20: mol_type = other DNA
ctgcgtggaagtctgtcaaa

SEQ ID NO: 40 - DNA, 20 bp, synthetic construct
  misc_feature 1..20: note = Primer
  source 1..20: mol_type = other DNA
ctatgccacagggcagtttt

SEQ ID NO: 41 - DNA, 20 bp, synthetic construct
  misc_feature 1..20: note = Primer
  source 1..20: mol_type = other DNA
tttgtcacgacctgcaatgc

SEQ ID NO: 42 - DNA, 20 bp, synthetic construct
  misc_feature 1..20: note = Primer
  source 1..20: mol_type = other DNA
aacaggcattgcacacatcg

SEQ ID NO: 43 - DNA, 20 bp, synthetic construct
  misc_feature 1..20: note = Primer
  source 1..20: mol_type = other DNA
acagcagcagcagcaatttc

SEQ ID NO: 44 - DNA, 20 bp, synthetic construct
  misc_feature 1..20: note = Primer
  source 1..20: mol_type = other DNA
tttccccaagccatcattgc

SEQ ID NO: 45 - DNA, 22 bp, synthetic construct
  misc_feature 1..22: note = Primer
  source 1..22: mol_type = other DNA
gatctccaaggccgagtatgat

SEQ ID NO: 46 - DNA, 20 bp, synthetic construct
  misc_feature 1..20: note = Primer
  source 1..20: mol_type = other DNA
cccattcataaaaccccagc